European Patent Application EP 4 324 850 A2, published February 21, 2024. Title: THERAPEUTIC ANTIGEN-BINDING MOLECULE WITH A FcRn-BINDING DOMAIN THAT PROMOTES ANTIGEN CLEARANCE. Applicant: CHUGAI SEIYAKU KABUSHIKI KAISHA. The sequence listing filed with the application follows.

SEQUENCE LISTING (29 sequences)

SEQ ID NO: 1 - protein, 447 aa, synthetic construct
  REGION 1..447: note = An artificially synthesized peptide sequence
QVQLQESGPGLVKPSETLSLTCAVSGHSISHDHAWSWVRQPPGEGLEWIGFISYSGITNYNPSLQGRVTISRDNSKNTLYLQMNSLRAEDTAVYYCARSLARTTAMDYWGEGTLVTVSSASTKGPSVFPLAPSSKSTSGGTAALGCLVKDYFPEPVTVSWNSGALTSGVHTFPAVLQSSGLYSLSSVVTVPSSSLGTQTYICNVNHKPSNTKVDKKVEPKSCDKTHTCPPCPAPELLGGPSVFLFPPKPKDTLMISRTPEVTCVVVDVSHEDPEVKFNWYVDGVEVHNAKTKPREEQYNSTYRVVSVLTVLHQDWLNGKEYKCKVSNKALPAPIEKTISKAKGQPREPQVYTLPPSRDELTKNQVSLTCLVKGFYPSDIAVEWESNGQPENNYKTTPPVLDSDGSFFLYSKLTVDKSRWQQGNVFSCSVMHEALHNHYTQKSLSLSP

SEQ ID NO: 2 - protein, 214 aa, synthetic construct [sequence omitted]

SEQ ID NO: 3 - protein, 214 aa, synthetic construct
  REGION 1..214: note = An artificially synthesized peptide sequence
DIQMTQSPSSLSASVGDSVTITCQASTDISSHLNWYQQKPGKAPELLIYYGSHLLSGVPSRFSGSGSGTDFTFTISSLEAEDAATYYCGQGNRLPYTFGQGTKVEIERTVAAPSVFIFPPSDEQLKSGTASVVCLLNNFYPREAKVQWKVDNALQSGNSQESVTEQDSKDSTYSLSSTLTLSKADYEKHKVYACEVTHQGLSSPVTKSFNRGEC

SEQ ID NO: 4 - protein, 447 aa, synthetic construct
  REGION 1..447: note = An artificially synthesized peptide sequence
QVQLQESGPGLVKPSETLSLTCAVSGHSISHDHAWSWVRQPPGEGLEWIGFISYSGITNYNPSLQGRVTISRDNSKNTLYLQMNSLRAEDTAVYYCARSLARTTAMDYWGEGTLVTVSSASTKGPSVFPLAPSSKSTSGGTAALGCLVKDYFPEPVTVSWNSGALTSGVHTFPAVLQSSGLYSLSSVVTVPSSSLGTQTYICNVNHKPSNTKVDKKVEPKSCDKTHTCPPCPAPELLGGPSVFLFPPKPKDTLYISRTPEVTCVVVDVSHEDPEVKFNWYVDGVEVHNAKTKPREEQYNSTYRVVSVLTVLHQDWLNGKEYKCKVSNKALPAPIEKTISKAKGQPREPQVYTLPPSRDELTKNQVSLTCLVKGFYPSDIAVEWESNGQPENNYKTTPPVLDSDGSFFLYSKLTVDKSRWQQGNVFSCSVMHEALHYHYTQKSLSLSP

SEQ ID NO: 5 - protein, 447 aa, synthetic construct
  REGION 1..447: note = An artificially synthesized peptide sequence
QVQLQESGPGLVKPSETLSLTCAVSGHSISHDHAWSWVRQPPGEGLEWIGFISYSGITNYNPSLQGRVTISRDNSKNTLYLQMNSLRAEDTAVYYCARSLARTTAMDYWGEGTLVTVSSASTKGPSVFPLAPSSKSTSGGTAALGCLVKDYFPEPVTVSWNSGALTSGVHTFPAVLQSSGLYSLSSVVTVPSSSLGTQTYICNVNHKPSNTKVDKKVEPKSCDKTHTCPPCPAPELLGGDSVFLFPPKPKDTLYISRTPEVTCVVVDVSHEDPEVKFNWYVDGVEVHNAKTKPREEQYNSTYRVVSVLTVLHQDWLNGKEYKCKVSNKALPAPIEKTISKAKGQPREPQVYTLPPSRDELTKNQVSLTCLVKGFYPSDIAVEWESNGQPENNYKTTPPVLDSDGSFFLYSKLTVDKSRWQQGNVFSCSVMHEALHYHYTQKSLSLSP

SEQ ID NO: 6 - protein, 447 aa, synthetic construct
  REGION 1..447: note = An artificially synthesized peptide sequence
QVQLQESGPGLVKPSETLSLTCAVSGHSISHDHAWSWVRQPPGEGLEWIGFISYSGITNYNPSLQGRVTISRDNSKNTLYLQMNSLRAEDTAVYYCARSLARTTAMDYWGEGTLVTVSSASTKGPSVFPLAPSSKSTSGGTAALGCLVKDYFPEPVTVSWNSGALTSGVHTFPAVLQSSGLYSLSSVVTVPSSSLGTQTYICNVNHKPSNTKVDKKVEPKSCDKTHTCPPCPAPELLGGPSVFLFPPKPKDTLYISRTPEVTCVVVDVSHEDPEVKFNWYVDGVEVHNAKTKPREEQYNSTYRVVSVLTVLHQDWLNGKEYKCKVSNKALPAPIEKTISKAKGQPREPQVYTLPPSRDELTKNQVSLTCLVKGFYPSDIAVEWESNGQPENNYKTTPPVLDSDGSFFLYSKLTVDKSRWQQGNVFSCSVMHEALHYHVTQKSLSLSP

SEQ ID NO: 7 - protein, 447 aa, synthetic construct
  REGION 1..447: note = An artificially synthesized peptide sequence
QVQLQESGPGLVKPSETLSLTCAVSGHSISHDHAWSWVRQPPGEGLEWIGFISYSGITNYNPSLQGRVTISRDNSKNTLYLQMNSLRAEDTAVYYCARSLARTTAMDYWGEGTLVTVSSASTKGPSVFPLAPSSKSTSGGTAALGCLVKDYFPEPVTVSWNSGALTSGVHTFPAVLQSSGLYSLSSVVTVPSSSLGTQTYICNVNHKPSNTKVDKKVEPKSCDKTHTCPPCPAPELLGGPSVFLFPPKPKDVLYISRTPEVTCVVVDVSHEDPEVKFNWYVDGVEVHNAKTKPREEQYNSTYRVVSVLQVLHADWLNGKEYKCKVSNKALPAPIEKTISKAKGQPREPQVYTLPPSRDELTKNQVSLTCLVKGFYPSDIAVEWESNGQPENNYKTTPPVLDSDGSFFLYSKLTVDKSRWQQGNVFSCSVMHEALHYHVTQKSLSLSP

SEQ ID NO: 8 - protein, 447 aa, synthetic construct
  REGION 1..447: note = An artificially synthesized peptide sequence
QVQLQESGPGLVKPSETLSLTCAVSGHSISHDHAWSWVRQPPGEGLEWIGFISYSGITNYNPSLQGRVTISRDNSKNTLYLQMNSLRAEDTAVYYCARSLARTTAMDYWGEGTLVTVSSASTKGPSVFPLAPSSKSTSGGTAALGCLVKDYFPEPVTVSWNSGALTSGVHTFPAVLQSSGLYSLSSVVTVPSSSLGTQTYICNVNHKPSNTKVDKKVEPKSCDKTHTCPPCPAPELRGGPKVFLFPPKPKDTLYITRTPEVTCVVVDVSHEDPEVKFNWYVDGVEVHNAKTKPREEQYNSTYRVVSVLTVLHQDWLNGKEYKCKVSNKALPAPIEKTISKAKGQPREPQVYTLPPSRDELTKNQVSLTCLVKGFYPSDIAVEWESNGQPENNYKTTPPVLDSDGSFFLYSKLTVDKSRWQQGNVFSCSVMHEALHYHVTRKELSLSP

SEQ ID NO: 9 - protein, 447 aa, synthetic construct
  REGION 1..447: note = An artificially synthesized peptide sequence
QVQLQESGPGLVKPSETLSLTCAVSGHSISHDHAWSWVRQPPGEGLEWIGFISYSGITNYNPSLQGRVTISRDNSKNTLYLQMNSLRAEDTAVYYCARSLARTTAMDYWGEGTLVTVSSASTKGPSVFPLAPSSKSTSGGTAALGCLVKDYFPEPVTVSWNSGALTSGVHTFPAVLQSSGLYSLSSVVTVPSSSLGTQTYICNVNHKPSNTKVDKKVEPKSCDKTHTCPPCPAPELRGGPKVFLFPPKPKDTLYITREPEVTCVVVDVSHEDPEVKFNWYVDGVEVHNAKTKPREEQYNSTYRVVSVLTVLHQDWLNGKEYKCKVSNKALPAPIEKTISKAKGQPREPQVYTLPPSRDELTKNQVSLTCLVKGFYPSDIAVEWESNGQPENNYKTTPPVLDSDGSFFLYSKLTVDKSRWQQGNVFSCSVMHEALHYHVTRKELSLSP

SEQ ID NO: 10 - protein, 447 aa, synthetic construct
  REGION 1..447: note = An artificially synthesized peptide sequence
QVQLQESGPGLVKPSETLSLTCAVSGHSISHDHAWSWVRQPPGEGLEWIGFISYSGITNYNPSLQGRVTISRDNSKNTLYLQMNSLRAEDTAVYYCARSLARTTAMDYWGEGTLVTVSSASTKGPSVFPLAPSSKSTSGGTAALGCLVKDYFPEPVTVSWNSGALTSGVHTFPAVLQSSGLYSLSSVVTVPSSSLGTQTYICNVNHKPSNTKVDKKVEPKSCDKTHTCPPCPAPELLGGPSVFLFPPKPKDTLMISRTPEVTCVVVDVSHEDPEVKFNWYVDGVEVHNAKTKPREEQYNSTYRVVSVLTVLHQDWLNGKEYKCKVSNKALPAPIEKTISKAKGQPREPQVYTLPPSRDELTKNQVSLTCLVKGFYPSDIAVEWESNGQPENNYKTTPPVLDSDGSFFLYSKLTVDKSRWQQGNVFSCSVLHEALHSHTTQKSLSLSP

SEQ ID NO: 11 - protein, 5 aa, synthetic construct
  REGION 1..5: note = An artificially synthesized peptide sequence
GGGGS

SEQ ID NO: 12 - protein, 464 aa, synthetic construct
  REGION 1..464: note = An artificially synthesized peptide sequence
QVQLQESGPGLVRPSQTLSLTCTVSGYSITSDHAWSWVRQPPGRGLEWIGYISYSGITTYNPSLKSRVTMLRDTSKNQFSLRLSSVTAADTAVYYCARSLARTTAMDYWGQGSLVTVSSASPTSPKVFPLSLCSTQPDGNVVIACLVQGFFPQEPLSVTWSESGQGVTARNFPPSQDASGDLYTTSSQLTLPATQCLAGKSVTCHVKHYTNPSQDVTVPCPVPSTPPTPSPSTPPTPSPSCCHPRLSLHRPALEDLLLGSEANLTCTLTGLRDASGVTFTWTPSSGKSAVQGPPERDLCGCYSVSSVLPGCAEPWNHGKTFTCTAAYPESKTPLTATLSKSGNTFRPEVHLLPPPSEELALNELVTLTCLARGFSPKDVLVRWLQGSQELPREKYLTWASRQEPSQGTTTFAVTSILRVAAEDWKKGDTFSCMVGHEALPLAFTQKTIDRLAGKEQKLISEEDL

SEQ ID NO: 13 - protein, 214 aa, synthetic construct [sequence omitted]

SEQ ID NO: 14 - protein, 451 aa, synthetic construct
  REGION 1..451: note = An artificially synthesized peptide sequence
QVQLVQSGAEVKKPGSSVKVSCKASGGTFSSYAISWVRQAPGQGLEWMGGIIPIFGTANYAQKFQGRVTITADESTSTAYMELSSLRSEDTAVYYCARPRWETAISSDAFDIWGQGTMVTVSSASTKGPSVFPLAPSSKSTSGGTAALGCLVKDYFPEPVTVSWNSGALTSGVHTFPAVLQSSGLYSLSSVVTVPSSSLGTQTYICNVNHKPSNTKVDKKVEPKSCDKTHTCPPCPAPELLGGPSVFLFPPKPKDTLMISRTPEVTCVVVDVSHEDPEVKFNWYVDGVEVHNAKTKPREEQYNSTYRVVSVLTVLHQDWLNGKEYKCKVSNKALPAPIEKTISKAKGQPREPQVYTLPPSRDELTKNQVSLTCLVKGFYPSDIAVEWESNGQPENNYKTTPPVLDSDGSFFLYSKLTVDKSRWQQGNVFSCSVMHEALHNHYTQKSLSLSP

SEQ ID NO: 15 - protein, 214 aa, synthetic construct
  REGION 1..214: note = An artificially synthesized peptide sequence
DIQMTQSPSSLSASVGDRVTITCRASQSISDDLNWYQQKPGKAPKLLIYEASNLQSGVPSRFSGSGSGTDFTLTISSLQPEDFATYYCQQHSSSPLTFGQGTKVEIKRTVAAPSVFIFPPSDEQLKSGTASVVCLLNNFYPREAKVQWKVDNALQSGNSQESVTEQDSKDSTYSLSSTLTLSKADYEKHKVYACEVTHQGLSSPVTKSFNRGEC

SEQ ID NO: 16 - protein, 451 aa, synthetic construct
  REGION 1..451: note = An artificially synthesized peptide sequence
QVQLVQSGAEVKKPGSSVKVSCKASGGTFSSYAISWVRQAPGQGLEWMGGIIPIFGTANYAQKFQGRVTITADESTSTAYMELSSLRSEDTAVYYCARPRWETAISSDAFDIWGQGTMVTVSSASTKGPSVFPLAPSSKSTSGGTAALGCLVKDYFPEPVTVSWNSGALTSGVHTFPAVLQSSGLYSLSSVVTVPSSSLGTQTYICNVNHKPSNTKVDKKVEPKSCDKTHTCPPCPAPELRGGPKVFLFPPKPKDTLMISRTPEVTCVVVDVSHEDPEVKFNWYVDGVEVHNAKTKPREEQYNSTYRVVSVLTVLHQDWLNGKEYKCKVSNKALPAPIEKTISKAKGQPREPQVYTLPPSRDELTKNQVSLTCLVKGFYPSDIAVEWESNGQPENNYKTTPPVLDSDGSFFLYSKLTVDKSRWQQGNVFSCSVMHEALHNHYTQKSLSLSP

SEQ ID NO: 17 - protein, 451 aa, synthetic construct
  REGION 1..451: note = An artificially synthesized peptide sequence
QVQLVQSGAEVKKPGSSVKVSCKASGGTFSSYAISWVRQAPGQGLEWMGGIIPIFGTANYAQKFQGRVTITADESTSTAYMELSSLRSEDTAVYYCARPRWETAISSDAFDIWGQGTMVTVSSASTKGPSVFPLAPSSKSTSGGTAALGCLVKDYFPEPVTVSWNSGALTSGVHTFPAVLQSSGLYSLSSVVTVPSSSLGTQTYICNVNHKPSNTKVDKKVEPKSCDKTHTCPPCPAPELRRGPKVFLFPPKPKDTLYITREPEVTCVVVDVSHEDPEVKFNWYVDGVEVHNAKTKPREEQYNSTYRVVSVLTVLHQDWLNGKEYKCKVSNKALPAPIEKTISKAKGQPREPQVYTLPPSRDELTKNQVSLTCLVKGFYPSDIAVEWESNGQPENNYKTTPPVLDSDGSFFLYSKLTVDKSRWQQGNVFSCSVMHEALHYHVTRKELSLSP

SEQ ID NO: 18 - protein, 543 aa, Homo sapiens
QVQLVQSGAEVKKPGASVKVSCKASGYTFTDYEMHWVRQAPGQGLEWMGALDPKTGDTAYSQKFKGRVTLTADKSTSTAYMELSSLTSEDTAVYYCTRFYSYTYWGQGTLVTVSSASTQSPSVFPLTRCCKNIPSNATSVTLGCLATGYFPEPVMVTWDTGSLNGTTMTLPATTLTLSGHYATISLLTVSGAWAKQMFTCRVAHTPSSTDWVDNKTFSVCSRDFTPPTVKILQSSCDGGGHFPPTIQLLCLVSGYTPGTINITWLEDGQVMDVDLSTASTTQEGELASTQSELTLSQKHWLSDRTYTCQVTYQGHTFEDSTKKCADSNPRGVSAYLSRPSPFDLFIRKSPTITCLVVDLAPSKGTVNLTWSRASGKPVNHSTRKEEKQRNGTLTVTSTLPVGTRDWIEGETYQCRVTHPHLPRALMRSTTKTSGPRAAPEVYAFATPEWPGSRDKRTLACLIQNFMPEDISVQWLHNEVQLPDARHSTTQPRKTKGSGFFVFSRLEVTRAEWEQKDEFICRAVHEAASPSQTVQRAVSVNPGK

SEQ ID NO: 19 - protein, 219 aa, Homo sapiens
DVVMTQSPLSLPVTPGEPASISCRSSQSLVHSNRNTYLHWYLQKPGQSPQLLIYKVSNRFSGVPDRFSGSGSGTDFTLKISRVEAEDVGVYYCSQNTHVPPTFGQGTKLEIKRTVAAPSVFIFPPSDEQLKSGTASVVCLLNNFYPREAKVQWKVDNALQSGNSQESVTEQDSKDSTYSLSSTLTLSKADYEKHKVYACEVTHQGLSSPVTKSFNRGEC

SEQ ID NO: 20 - protein, 443 aa, synthetic construct
  REGION 1..443: note = An artificially synthesized peptide sequence
QSLEESGGRLVTPGTPLTLTCTASGFSLSSYHMSWVRQAPGKGLEWIGVINSAGNTYYASWAKGRFTVSKTSTTVDLNLTSLTTEDTATYFCARYVFSSGSHDIWGPGTLVTVSSASTKGPSVFPLAPSSKSTSGGTAALGCLVKDYFPEPVTVSWNSGALTSGVHTFPAVLQSSGLYSLSSVVTVPSSSLGTQTYICNVNHKPSNTKVDKKVEPKSCDKTHTCPPCPAPELLGGPSVFLFPPKPKDTLMISRTPEVTCVVVDVSHEDPEVKFNWYVDGVEVHNAKTKPREEQYNSTYRVVSVLTVLHQDWLNGKEYKCKVSNKALPAPIEKTISKAKGQPREPQVYTLPPSREEMTKNQVSLTCLVKGFYPSDIAVEWESNGQPENNYKTTPPVLDSDGSFFLYSKLTVDKSRWQQGNVFSCSVMHEALHNHYTQKSLSLSP

SEQ ID NO: 21 - protein, 217 aa, synthetic construct
  REGION 1..217: note = An artificially synthesized peptide sequence
AYDMTQTPASVEVAVGGTVTIKCQASQSIGSWLAWYQQKPGQPPKELIYGTSTLESGVPSRFIGSGSGTEFTLTISGVECADAATYYCQQGYSEDNIDNAFGGGTEVVVKRTVAAPSVFIFPPSDEQLKSGTASVVCLLNNFYPREAKVQWKVDNALQSGNSQESVTEQDSKDSTYSLSSTLTLSKADYEKHKVYACEVTHQGLSSPVTKSFNRGEC

SEQ ID NO: 22 - protein, 32 aa, synthetic construct
  REGION 1..32: note = An artificially synthesized peptide sequence
VDDAPGNSQQATPKDNEISTFHNLGNVHSPLK

SEQ ID NO: 23 - protein, 443 aa, synthetic construct
  REGION 1..443: note = An artificially synthesized peptide sequence
QSLEESGGRLVTPGTPLTLTCTASGFSLSSYHMSWVRQAPGKGLEWIGVINSAGNTYYASWAKGRFTVSKTSTTVDLNLTSLTTEDTATYFCARYVFSSGSHDIWGPGTLVTVSSASTKGPSVFPLAPSSKSTSGGTAALGCLVKDYFPEPVTVSWNSGALTSGVHTFPAVLQSSGLYSLSSVVTVPSSSLGTQTYICNVNHKPSNTKVDKKVEPKSCDKTHTCPPCPAPELRGGPKVFLFPPKPKDTLMISRTPEVTCVVVDVSHEDPEVKFNWYVDGVEVHNAKTKPREEQYNSTYRVVSVLTVLHQDWLNGKEYKCKVSNKALPAPIEKTISKAKGQPREPQVYTLPPSRDELTKNQVSLTCLVKGFYPSDIAVEWESNGQPENNYKTTPPVLDSDGSFFLYSKLTVDKSRWQQGNVFSCSVMHEALHNHYTQKSLSLSP

SEQ ID NO: 24 - protein, 443 aa, synthetic construct
  REGION 1..443: note = An artificially synthesized peptide sequence
QSLEESGGRLVTPGTPLTLTCTASGFSLSSYHMSWVRQAPGKGLEWIGVINSAGNTYYASWAKGRFTVSKTSTTVDLNLTSLTTEDTATYFCARYVFSSGSHDIWGPGTLVTVSSASTKGPSVFPLAPSSKSTSGGTAALGCLVKDYFPEPVTVSWNSGALTSGVHTFPAVLQSSGLYSLSSVVTVPSSSLGTQTYICNVNHKPSNTKVDKKVEPKSCDKTHTCPPCPAPELRRGPKVFLFPPKPKDTLYITREPEVTCVVVDVSHEDPEVKFNWYVDGVEVHNAKTKPREEQYNSTYRVVSVLTVLHQDWLNGKEYKCKVSNKALPAPIEKTISKAKGQPREPQVYTLPPSRDELTKNQVSLTCLVKGFYPSDIAVEWESNGQPENNYKTTPPVLDSDGSFFLYSKLTVDKSRWQQGNVFSCSVMHEALHYHVTRKELSLSP

SEQ ID NO: 25 - protein, 543 aa, synthetic construct
  REGION 1..543: note = An artificially synthesized peptide sequence
QVQLVQSGAEVKKPGASVKVSCKASGYTFTDYEMHWVRQAPGQGLEWMGALDPKTGDTAYSQKFKGRVTLTADKSTSTAYMELSSLTSEDTAVYYCTRFYSYTYWGQGTLVTVSSASTQSPSVFPLTRCCKNIPSDATSVTLGCLATGYFPEPVMVTWDTGSLDGTTMTLPATTLTLSGHYATISLLTVSGAWAKQMFTCRVAHTPSSTDWVDDKTFSVCSRDFTPPTVKILQSSCDGGGHFPPTIQLLCLVSGYTPGTIDITWLEDGQVMDVDLSTASTTQEGELASTQSELTLSQKHWLSDRTYTCQVTYQGHTFEDSTKKCADSNPRGVSAYLSRPSPFDLFIRKSPTITCLVVDLAPSKGTVDLTWSRASGKPVDHSTRKEEKQRNGTLTVTSTLPVGTRDWIEGETYQCRVTHPHLPRALMRSTTKTSGPRAAPEVYAFATPEWPGSRDKRTLACLIQNFMPEDISVQWLHNEVQLPDARHSTTQPRKTKGSGFFVFSRLEVTRAEWEQKDEFICRAVHEAASPSQTVQRAVSVNPGK

SEQ ID NO: 26 - protein, 545 aa, Homo sapiens
QPPPPPPDATCHQVRSFFQRLQPGLKWVPETPVPGSDLQVCLPKGPTCCSRKMEEKYQLTARLNMEQLLQSASMELKFLIIQNAAVFQEAFEIVVRHAKNYTNAMFKNNYPSLTPQAFEFVGEFFTDVSLYILGSDINVDDMVNELFDSLFPVIYTQLMNPGLPDSALDINECLRGARRDLKVFGNFPKLIMTQVSKSLQVTRIFLQALNLGIEVINTTDHLKFSKDCGRMLTRMWYCSYCQGLMMVKPCGGYCNVVMQGCMAGVVEIDKYWREYILSLEELVNGMYRIYDMENVLLGLFSTIHDSIQYVQKNAGKLTTTIGKLCAHSQQRQYRSAYYPEDLFIDKKVLKVAHVEHEETLSSRRRELIQKLKSFISFYSALPGYICSHSPVAENDTLCWNGQELVERYSQKAARNGMKNQFNLHELKMKGPEPVVSQIIDKLKHINQLLRTMSMPKGRVLDKNLDEEGFEAGDCGDDEDECIGGAGDGMIKVKNQLRFLAELAYDLDVDDAPGNSQQATPKDNEISTFHNLGNVHSPLKHHHHHH

SEQ ID NO: 27 - protein, 365 aa, Homo sapiens
MGVPRPQPWALGLLLFLLPGSLGAESHLSLLYHLTAVSSPAPGTPAFWVSGWLGPQQYLSYNSLRGEAEPCGAWVWENQVSWYWEKETTDLRIKEKLFLEAFKALGGKGPYTLQGLLGCELGPDNTSVPTAKFALNGEEFMNFDLKQGTWGGDWPEALAISQRWQQQDKAANKELTFLLFSCPHRLREHLERGRGNLEWKEPPSMRLKARPSSPGFSVLTCSAFSFYPPELQLRFLRNGLAAGTGQGDFGPNSDGSFHASSSLTVKSGDEHHYCCIVQHAGLAQPLRVELESPAKSSVLVVGIVIGVLLLTAAAVGGALLWRRMRSGLPAPWISLRGDDTGVLLPTPGEAQDADLKDVNVIPATA

SEQ ID NO: 28 - protein, 119 aa, Homo sapiens
MSRSVALAVLALLSLSGLEAIQRTPKIQVYSRHPAENGKSNFLNCYVSGFHPSDIEVDLLKNGERIEKVEHSDLSFSKDWSFYLLYYTEFTPTEKDEYACRVNHVTLSQPKIVKWDRDM

SEQ ID NO: 29 - protein, 8 aa, synthetic construct
  REGION 1..8: note = An artificially synthesized peptide sequence
DYKDDDDK